European Patent Specification EP 3 662 915 B1, published February 22, 2023. Title: Stem cells for transplantation and manufacturing method therefor. Applicant: National Center of Neurology and Psychiatry. The sequence listing filed with the application follows.

SEQUENCE LISTING (14 sequences)

SEQ ID NO: 1 - protein, 178 aa, Homo sapiens
  human IL-10
MHSSALLCCLVLLTGVRASPGQGTQSENSCTHFPGNLPNMLRDLRDAFSRVKTFFQMKDQLDNLLLKESLLEDFKGYLGCQALSEMIQFYLEEVMPQAENQDPDIKAHVNSLGENLKTLRLRLRRCHRFLPCENKSKAVEQVKNAFNKLQEKGIYKAMSEFDIFINYIEAYMTMKIRN

SEQ ID NO: 2 - DNA, 537 bp, Homo sapiens
  human IL-10 cDNA
atgcacagctcagcactgctctgttgcctggtcctcctgactggggtgagggccagcccaggccagggcacccagtctgagaacagctgcacccacttcccaggcaacctgcctaacatgcttcgagatctccgagatgccttcagcagagtgaagactttctttcaaatgaaggatcagctggacaacttgttgttaaaggagtccttgctggaggactttaagggttacctgggttgccaagccttgtctgagatgatccagttttacctggaggaggtgatgccccaagctgagaaccaagacccagacatcaaggcgcatgtgaactccctgggggagaacctgaagaccctcaggctgaggctacggcgctgtcatcgatttcttccctgtgaaaacaagagcaaggccgtggagcaggtgaagaatgcctttaataagctccaagagaaaggcatctacaaagccatgagtgagtttgacatcttcatcaactacatagaagcctacatgacaatgaagatacgaaactga

SEQ ID NO: 3 - protein, 178 aa, Mus musculus
  mouse IL-10
MPGSALLCCLLLLTGMRISRGQYSREDNNCTHFPVGQSHMLLELRTAFSQVKTFFQTKDQLDNILLTDSLMQDFKGYLGCQALSEMIQFYLVEVMPQAEKHGPEIKEHLNSLGEKLKTLRMRLRRCHRFLPCENKSKAVEQVKSDFNKLQDQGVYKAMNEFDIFINCIEAYMMIKMKS

SEQ ID NO: 4 - DNA, 537 bp, Mus musculus
  mouse IL-10 cDNA
atgcctggctcagcactgctatgctgcctgctcttactgactggcatgaggatcagcaggggccagtacagccgggaagacaataactgcacccacttcccagtcggccagagccacatgctcctagagctgcggactgccttcagccaggtgaagactttctttcaaacaaaggaccagctggacaacatactgctaaccgactccttaatgcaggactttaagggttacttgggttgccaagccttatcggaaatgatccagttttacctggtagaagtgatgccccaggcagagaagcatggcccagaaatcaaggagcatttgaattccctgggtgagaagctgaagaccctcaggatgcggctgaggcgctgtcatcgatttctcccctgtgaaaataagagcaaggcagtggagcaggtgaagagtgattttaataagctccaagaccaaggtgtctacaaggccatgaatgaatttgacatcttcatcaactgcatagaagcatacatgatgatcaaaatgaaaagctaa

SEQ ID NO: 5 - protein, 178 aa, Rattus norvegicus
  Rat IL-10
MPGSALLCCLLLLAGVKTSKGHSIRGDNNCTHFPVSQTHMLRELRAAFSQVKTFFQKKDQLDNILLTDSLLQDFKGYLGCQALSEMIKFYLVEVMPQAENHGPEIKEHLNSLGEKLKTLWIQLRRCHRFLPCENKSKAVEQVKNDFNKLQDKGVYKAMNEFDIFINCIEAYVTLKMKN

SEQ ID NO: 6 - DNA, 538 bp, Rattus norvegicus
  Rat IL-10 cDNA
catgcctggctcagcactgctatgttgcctgctcttactggctggagtgaagaccagcaaaggccattccatccggggtgacaataactgcacccacttcccagtcagccagacccacatgctccgagagctgagggctgccttcagtcaagtgaagactttctttcaaaagaaggaccagctggacaacatactgctgacagattccttactgcaggactttaagggttacttgggttgccaagccttgtcagaaatgatcaagttttacctggtagaagtgatgccccaggcagagaaccatggcccagaaatcaaggagcatttgaattccctgggagagaagctgaagaccctctggatacagctgcgacgctgtcatcgatttctcccctgtgagaataaaagcaaggcagtggagcaggtgaagaatgattttaataagctccaagacaaaggtgtctacaaggccatgaatgagtttgacatcttcatcaactgcatagaagcctacgtgacactcaaaatgaaaaattga

SEQ ID NO: 7 - protein, 181 aa, Canis lupus familiaris
  dog IL-10
MHGSALLCCCLVLLAGVGASRHQSTLLEDDCTHFPASLPHMLRELRAAFGRVKIFFQMKDKLDNILLTGSLLEDFKSYLGCQALSEMIQFYLEEVMPRAENHDPDIKNHVNSLGEKLKTLRLRLRLRRCHRFLPCENKSKAVEQVKSAFSKLQEKGVYKAMSEFDIFINYIETYMTMRMKI

SEQ ID NO: 8 - DNA, 546 bp, Canis lupus familiaris
  dog IL-10 cDNA
atgcatggctcagcactgctctgttgctgcctggtcctcctggccggggtgggagccagccgacaccagagcaccctacttgaggacgactgcacccacttcccagccagcctgccccacatgctccgagagctccgagctgccttcgggagggtgaagatcttctttcaaatgaaggacaagctggacaacatactgctgaccgggtccctgctggaggactttaagagttacctgggttgccaagccctgtcggagatgatccagttttacttggaggaggtgatgccccgggctgagaaccacgacccagacatcaagaaccacgtgaactccctgggagagaagctcaagaccctcaggctgagactgaggctgcgacgctgtcaccgatttcttccctgtgagaataagagcaaggcggtggagcaggtgaagagcgcatttagtaagctccaggagaaaggtgtctacaaagccatgagtgagtttgacatcttcatcaactacatagaaacctacatgacaatgaggatgaaaatctga

SEQ ID NO: 9 - protein, 178 aa, Pan troglodytes
  chimpanzee IL-10
MHSSALLCCLVLLTGVRASPGQGTQSENSCTHFPGNLPNMLRDLRDAFSRVKTFFQMKDQLDNLLLKESLLEDFKGYLGCQALSEMIQFYLEEVMPQAENQDPDIKVHVNSLGENLKTLRLRLRRCHRFLPCENKSKAVEQVKNAFNKLQEKGIYKAMSEFDIFINYIEAYMTMKIRN

SEQ ID NO: 10 - DNA, 537 bp, Pan troglodytes
  chimpanzee IL-10 cDNA
atgcacagctcagcactgctctgttgcctggtcctcctgactggggtgagggccagcccaggccagggcacccagtctgagaacagctgcacccacttcccaggcaacctgcctaacatgcttcgagatctccgagatgccttcagcagagtgaagactttctttcaaatgaaggatcagctggacaacttgctgttaaaggagtccttgctggaggactttaagggttacctgggttgccaagccttgtctgagatgatccagttttacctggaggaggtgatgccccaagctgagaaccaagacccagacatcaaggtgcatgtgaactccctgggggagaacctgaagaccctcaggctgaggctacggcgctgtcatcgatttcttccctgtgaaaacaagagcaaggccgtggagcaggtgaagaatgcctttaataagctccaagagaaaggcatctacaaagccatgagtgagtttgacatcttcatcaactacatagaagcctacatgacaatgaagatacgaaactga

SEQ ID NO: 11 - protein, 178 aa, Bos taurus
  crummy IL-10
MHSSALLCCLVFLAGVAASRDASTLSDSSCIHLPTSLPHMLRELRAAFGEAKTFFQMKDQLHSLLLTQSLLDDFKGYLGCQALSEMIQFYLEEVMPQAENHGPDIKEHVNSLGEKLKTLRLRLRRCHRFLPCENKSKAVEKVKRVFSELQERGVYKAMSEFDIFINYIETYMTTKMQK

SEQ ID NO: 12 - DNA, 537 bp, Bos taurus
  crummy IL-10 cDNA
atgcatagctcagcactactctgttgcctggtcttcctggctggggtggcagccagccgagatgcgagcaccctgtctgacagcagctgtatccacttgccaaccagcctgccccacatgctgcgggagctccgagctgccttcggcgaggcgaagactttctttcaaatgaaggaccaactgcacagcttactgttgacccagtctctgctggatgactttaagggttacctgggttgccaagccttgtcggaaatgatccagttttacctggaagaggtgatgccacaggctgagaaccacgggcctgacatcaaggagcacgtgaactcactgggggagaagctgaagaccctgcggctgcggctgcggcgctgtcatcgctttctgccctgcgaaaacaagagcaaggcggtggagaaggtgaagagagtcttcagtgagctccaagagaggggtgtctacaaagccatgagtgagtttgacatcttcatcaactacatagaaacctacatgacaacgaagatgcaaaagtga

SEQ ID NO: 13 - DNA, 34 bp, Artificial
  primer
cgcggatccatgcctggctcagcactgctatgct

SEQ ID NO: 14 - DNA, 31 bp, Artificial
  primer
gaggatcctcttagcttttcattttgatcat